European Patent Specification EP 3 583 215 B1, published March 19, 2025. Title: System und Verfahren zur Zelltyp-spezifischen Translation von RNA-Molekülen in Eukaryoten. Applicant: aReNA-Bio GbR. The sequence listing filed with the application follows.

SEQUENCE LISTING (7 sequences)

SEQ ID NO: 1 - DNA, 402 bp, Hepatitis C virus
gccagcccccgattgggggcgacactccaccatagatcactcccctgtgaggaactactgtcttcacgcagaaagcgtctagccatggcgttagtatgagtgtcgtgcagcctccaggaccccccctcccgggagagccatagtggtctgcggaaccggtgagtacaccggaattgccaggacgaccgggtcctttcttggatcaacccgctcaatgcctggagatttgggcgtgcccccgcgagactgctagccgagtagtgttgggtcgcgaaaggccttgtggtactgcctgatagggtgcttgcgagtgccccgggaggtctcgtagaccgtgcaccatgagcacgaatcctaaacctcaaagaaaaaccaaacgtaacaccaaccgccgcccacagg

SEQ ID NO: 2 - DNA, 459 bp, Artificial Sequence
  IRES-Sequenz (Position 6 in Abb.6) mit 3 stabilisierenden Elementen
gccagcccccgattggggggccagcccccgattggggggccagcccccgattggggggccagcccccgattgggggcgacactccaccatagatcactcccctgtgaggaactactgtcttcacgcagaaagcgtctagccatggcgttagtatgagtgtcgtgcagcctccaggaccccccctcccgggagagccatagtggtctgcggaaccggtgagtacaccggaattgccaggacgaccgggtcctttcttggatcaacccgctcaatgcctggagatttgggcgtgcccccgcgagactgctagccgagtagtgttgggtcgcgaaaggccttgtggtactgcctgatagggtgcttgcgagtgccccgggaggtctcgtagaccgtgcaccatgagcacgaatcctaaacctcaaagaaaaaccaaacgtaacaccaaccgccgcccacagg

SEQ ID NO: 3 - DNA, 498 bp, Artificial Sequence
  Primäre IRES-Sequenz (Position 6 in Abb.8) mit 3 stabilisierenden Elementen (Position 5 in Abb. 8, unterstrichen) und und Linker (Position 4a in Abbildung 8, eingerahmt)
ataaataaataaaataaataaataaaataaataaataaagccagcccccgattggggggccagcccccgattggggggccagcccccgattggggggccagcccccgattgggggcgacactccaccatagatcactcccctgtgaggaactactgtcttcacgcagaaagcgtctagccatggcgttagtatgagtgtcgtgcagcctccaggaccccccctcccgggagagccatagtggtctgcggaaccggtgagtacaccggaattgccaggacgaccgggtcctttcttggatcaacccgctcaatgcctggagatttgggcgtgcccccgcgagactgctagccgagtagtgttgggtcgcgaaaggccttgtggtactgcctgatagggtgcttgcgagtgccccgggaggtctcgtagaccgtgcaccatgagcacgaatcctaaacctcaaagaaaaaccaaacgtaacaccaaccgccgcccacagg

SEQ ID NO: 4 - DNA, 507 bp, Artificial Sequence
  Primäre IRES-Sequenz (Position 6 in Abb.10) mit 3 stabilisierenden Elementen (Position 5 in Abb. 10, unterstrichen), Linker (Position 4a in Abbildung 8, eingerahmt) und und Blocker
cccaacactataaataaataaaataaataaataaaataaataaataaagccagcccccgattggggggccagcccccgattggggggccagcccccgattggggggccagcccccgattgggggcgacactccaccatagatcactcccctgtgaggaactactgtcttcacgcagaaagcgtctagccatggcgttagtatgagtgtcgtgcagcctccaggaccccccctcccgggagagccatagtggtctgcggaaccggtgagtacaccggaattgccaggacgaccgggtcctttcttggatcaacccgctcaatgcctggagatttgggcgtgcccccgcgagactgctagccgagtagtgttgggtcgcgaaaggccttgtggtactgcctgatagggtgcttgcgagtgccccgggaggtctcgtagaccgtgcaccatgagcacgaatcctaaacctcaaagaaaaaccaaacgtaacaccaaccgccgcccacagg

SEQ ID NO: 5 - DNA, 1619 bp, Artificial Sequence
  Nukleotidsequenz des funktionalen Systems zur selektiven Expression von Zielsequenzen in de-finierten Zelltypen (Keratin 13)
acgcaccggtcggcctcctcccagctggcaagagccacccccgaaaccacctccatagctggcagaggagctctgcaggcggaggctcatgaattcgttatgttatgaccttgctcgtcaagaagacagttatgttattaaaagtcaggtcggatcaagccatagtacggaaaaaactatgctacctgtgagccccgtccaaggacgtgcggccgctaaaagaagtcaggccatcacaaatgccacagcttgagtaaactgtgcagcctgtagctccacctgagaaggtgtaaaaaagttatgttatggatcccccccctaacgttactggccgaagccgcttggaataaggccggtgtgcgtttgtctatatgttattttccaccatattgccgtcttttggcaatgtgagggcccggaaacctggccctgtcttcttgacgagcattcctaggggtctttcccctctcgccaaaggaatgcaaggtctgttgaatgtcgtgaaggaagcagttcctctggaagcttcttgaagacaaacaacgtctgtagcgaccctttgcaggcagcggaaccccccacctggcgacaggtgcctctgcggccaaaagccacgtgtataagatacacctgcaaaggcggcacaaccccagtgccacgttgtgagttggatagttgtggaaagagtcaaatggctctcctcaagcgtattcaacaaggggctgaaggatgcccagaaggtaccccattgtatgggatctgatctggggcctcggtgcacatgctttacatgtgtttagtcgaggttaaaaaacgtctaggccccccgaaccacggggacgtggttttcctttgaaaaacacgatgataatatggccacaaccatgtctagaatggtgagcaagggcgaggagctgttcaccggggtggtgcccatcctggtcgagctggacggcgacgtaaacggccacaagttcagcgtgtccggcgagggcgagggcgatgccacctacggcaagctgaccctgaagttcatctgcaccaccggcaagctgcccgtgccctggcccaccctcgtgaccaccctgacctacggcgtgcagtgcttcagccgctaccccgaccacatgaagcagcacgacttcttcaagtccgccatgcccgaaggctacgtccaggagcgcaccatcttcttcaaggacgacggcaactacaagacccgcgccgaggtgaagttcgagggcgacaccctggtgaaccgcatcgagctgaagggcatcgacttcaaggaggacggcaacatcctggggcacaagctggagtacaactacaacagccacaacgtctatatcatggccgacaagcagaagaacggcatcaaggtgaacttcaagatccgccacaacatcgaggacggcagcgtgcagctcgccgaccactaccagcagaacacccccatcggcgacggccccgtgctgctgcccgacaaccactacctgagcacccagtccgccctgagcaaagaccccaacgagaagcgcgatcacatggtcctgctggagttcgtgaccgccgccgggatcactctcggcatggacgagctgtacaagtaagtcgac

SEQ ID NO: 6 - DNA, 2164 bp, Artificial Sequence
  Nukleotidsequenz des funktionalen Systems mit alternativer antisense-Sequenz zur selektiven Expression von Zielsequenzen in definierten Zelltypen
acgcaccggttgatgtcggcctccacgctctggcgcagggccagctcattctcatacttgagcctgaagtcgtccgcagccagcctggcattgtcaatctccaggatgacccggttgttttcaatggtggcggtcaggatcttgtcccggagctcttcaatggtcttgtagtaggggctgtagtcccgctcagggctagctgggctctgcttcaggtgccagtcacggatcttcacctccaggtcagcgttggcctcctccagggcgcgcaccttctccaggtaggaagccaggcggtcgttgaggttctgcatggtgatcttctcattgccagtgaggaggccgccatcacaagcaccaaagtcaacaaagccaccagcaaaacccccaccaaagccacctccaaggccacctccatagccacctccaaggccacctccatagccacctccaaagccactaccagcccctccaccaaaaccacagctcacgccgcctccatagcccccagctgatcccccagacacaaaccgagttgaacaggtagagacaccacggcctcctcccagctggcaagagccacccccgaaaccacctccatagctggcagaggagctctgcaggcggaggctcatgaattcgttatgttatgaccttgctcgtcaagaagacagttatgttattaaaagtcaggtcggatcaagccatagtacggaaaaaactatgctacctgtgagccccgtccaaggacgtgcggccgctaaaagaagtcaggccatcacaaatgccacagcttgagtaaactgtgcagcctgtagctccacctgagaaggtgtaaaaaagttatgttatggatcccccccctaacgttactggccgaagccgcttggaataaggccggtgtgcgtttgtctatatgttattttccaccatattgccgtcttttggcaatgtgagggcccggaaacctggccctgtcttcttgacgagcattcctaggggtctttcccctctcgccaaaggaatgcaaggtctgttgaatgtcgtgaaggaagcagttcctctggaagcttcttgaagacaaacaacgtctgtagcgaccctttgcaggcagcggaaccccccacctggcgacaggtgcctctgcggccaaaagccacgtgtataagatacacctgcaaaggcggcacaaccccagtgccacgttgtgagttggatagttgtggaaagagtcaaatggctctcctcaagcgtattcaacaaggggctgaaggatgcccagaaggtaccccattgtatgggatctgatctggggcctcggtgcacatgctttacatgtgtttagtcgaggttaaaaaacgtctaggccccccgaaccacggggacgtggttttcctttgaaaaacacgatgataatatggccacaaccatgtctagaatggtgagcaagggcgaggagctgttcaccggggtggtgcccatcctggtcgagctggacggcgacgtaaacggccacaagttcagcgtgtccggcgagggcgagggcgatgccacctacggcaagctgaccctgaagttcatctgcaccaccggcaagctgcccgtgccctggcccaccctcgtgaccaccctgacctacggcgtgcagtgcttcagccgctaccccgaccacatgaagcagcacgacttcttcaagtccgccatgcccgaaggctacgtccaggagcgcaccatcttcttcaaggacgacggcaactacaagacccgcgccgaggtgaagttcgagggcgacaccctggtgaaccgcatcgagctgaagggcatcgacttcaaggaggacggcaacatcctggggcacaagctggagtacaactacaacagccacaacgtctatatcatggccgacaagcagaagaacggcatcaaggtgaacttcaagatccgccacaacatcgaggacggcagcgtgcagctcgccgaccactaccagcagaacacccccatcggcgacggccccgtgctgctgcccgacaaccactacctgagcacccagtccgccctgagcaaagaccccaacgagaagcgcgatcacatggtcctgctggagttcgtgaccgccgccgggatcactctcggcatggacgagctgtacaagtaagtcgac

SEQ ID NO: 7 - DNA, 2175 bp, Artificial Sequence
  Nukleotidsequenz des funktionalen Systems mit alternativer antisense-Sequenz und alternativer Blocker-Sequenz zur selektiven Expression von Zielsequenzen in definierten Zelltypen
acgcaccggttgatgtcggcctccacgctctggcgcagggccagctcattctcatacttgagcctgaagtcgtccgcagccagcctggcattgtcaatctccaggatgacccggttgttttcaatggtggcggtcaggatcttgtcccggagctcttcaatggtcttgtagtaggggctgtagtcccgctcagggctagctgggctctgcttcaggtgccagtcacggatcttcacctccaggtcagcgttggcctcctccagggcgcgcaccttctccaggtaggaagccaggcggtcgttgaggttctgcatggtgatcttctcattgccagtgaggaggccgccatcacaagcaccaaagtcaacaaagccaccagcaaaacccccaccaaagccacctccaaggccacctccatagccacctccaaggccacctccatagccacctccaaagccactaccagcccctccaccaaaaccacagctcacgccgcctccatagcccccagctgatcccccagacacaaaccgagttgaacaggtagagacaccacggcctcctcccagctggcaagagccacccccgaaaccacctccatagctggcagaggagctctgcaggcggaggctcatgaattcgttatgttatgaactgcttccttcacgacattcaacagaccttgttatgttattaaaagtcaggtcggatcaagccatagtacggaaaaaactatgctacctgtgagccccgtccaaggacgtgcggccgctaaaagaagtcaggccatcacaaatgccacagcttgagtaaactgtgcagcctgtagctccacctgagaaggtgtaaaaaagttatgttatggatcccccccctaacgttactggccgaagccgcttggaataaggccggtgtgcgtttgtctatatgttattttccaccatattgccgtcttttggcaatgtgagggcccggaaacctggccctgtcttcttgacgagcattcctaggggtctttcccctctcgccaaaggaatgcaaggtctgttgaatgtcgtgaaggaagcagttcctctggaagcttcttgaagacaaacaacgtctgtagcgaccctttgcaggcagcggaaccccccacctggcgacaggtgcctctgcggccaaaagccacgtgtataagatacacctgcaaaggcggcacaaccccagtgccacgttgtgagttggatagttgtggaaagagtcaaatggctctcctcaagcgtattcaacaaggggctgaaggatgcccagaaggtaccccattgtatgggatctgatctggggcctcggtgcacatgctttacatgtgtttagtcgaggttaaaaaacgtctaggccccccgaaccacggggacgtggttttcctttgaaaaacacgatgataatatggccacaaccatgtctagaatggtgagcaagggcgaggagctgttcaccggggtggtgcccatcctggtcgagctggacggcgacgtaaacggccacaagttcagcgtgtccggcgagggcgagggcgatgccacctacggcaagctgaccctgaagttcatctgcaccaccggcaagctgcccgtgccctggcccaccctcgtgaccaccctgacctacggcgtgcagtgcttcagccgctaccccgaccacatgaagcagcacgacttcttcaagtccgccatgcccgaaggctacgtccaggagcgcaccatcttcttcaaggacgacggcaactacaagacccgcgccgaggtgaagttcgagggcgacaccctggtgaaccgcatcgagctgaagggcatcgacttcaaggaggacggcaacatcctggggcacaagctggagtacaactacaacagccacaacgtctatatcatggccgacaagcagaagaacggcatcaaggtgaacttcaagatccgccacaacatcgaggacggcagcgtgcagctcgccgaccactaccagcagaacacccccatcggcgacggccccgtgctgctgcccgacaaccactacctgagcacccagtccgccctgagcaaagaccccaacgagaagcgcgatcacatggtcctgctggagttcgtgaccgccgccgggatcactctcggcatggacgagctgtacaagtaagtcgac